European Patent Specification EP 3 970 796 B1, published August 20, 2025. Title: A Composition for Preventing or Treating Neurotrophic Keratitis comprising a PACAP Peptide or a Stabilized Peptide of PACAP. Applicant: Senju Pharmaceutical Co., Ltd. The sequence listing filed with the application follows.

SEQUENCE LISTING (44 sequences)

SEQ ID NO: 1 - protein, 38 aa, Homo sapiens
HSDGIFTDSYSRYRKQMAVKKYLAAVLGKRYKQRVKNK

SEQ ID NO: 2 - protein, 27 aa, Homo sapiens
HSDGIFTDSYSRYRKQMAVKKYLAAVL

SEQ ID NO: 3 - protein, 27 aa, Artificial Sequence
  Synthetic Peptide
  MISC_FEATURE (2)..(2): Xaa is neutral amino acid
  MUTAGEN (9)..(9): Xaa is neutral amino acid
  MUTAGEN (11)..(11): Xaa is neutral amino acid
  MUTAGEN (15)..(15): Xaa is basic amino acid
  MUTAGEN (16)..(16): Xaa is neutral amino acid or amino acid wherein amide of glutamine is substituted with tetrazole
  MUTAGEN (17)..(17): Xaa is non-polar amino acid
  MUTAGEN (19)..(19): Xaa is non-polar amino acid
  MUTAGEN (20)..(20): Xaa is basic amino acid
  MUTAGEN (21)..(21): Xaa is basic amino acid
  MUTAGEN (27)..(27): Xaa is non-polar amino acid
HXDGIFTDXYXRYRXXXAXXXYLAAVX

SEQ ID NO: 4 - protein, 27 aa, Artificial Sequence
  Syntehtic Peptide
  MOD_RES (1)..(1): ACETYLATION
HSDGIFTDSYSRYRKQMAVKKYLAAVL

SEQ ID NO: 5 - protein, 27 aa, Artificial Sequence
  Syntehtic Peptide
  MUTAGEN (3)..(3): Xaa is amino acid wherein carboxy group of asparatic acid is substituted with tetrazole
HSXGIFTDSYSRYRKQMAVKKYLAAVL

SEQ ID NO: 6 - protein, 27 aa, Artificial Sequence
  Syntehtic Peptide
  MUTAGEN (8)..(8): Xaa is amino acid wherein carboxy group of asparatic acid is substituted with tetrazole
HSDGIFTXSYSRYRKQMAVKKYLAAVL

SEQ ID NO: 7 - protein, 27 aa, Artificial Sequence
  Syntehtic Peptide
  MUTAGEN (3)..(3): Xaa is amino acid wherein carboxy group of asparatic acid is substituted with tetrazole
  MUTAGEN (8)..(8): Xaa is amino acid wherein carboxy group of asparatic acid is substituted with tetrazole
HSXGIFTXSYSRYRKQMAVKKYLAAVL

SEQ ID NO: 8 - protein, 27 aa, Artificial Sequence
  Syntehtic Peptide
  MUTAGEN (3)..(3): Xaa is amino acid wherein carboxy group of asparatic acid is substituted with tetrazole
  MUTAGEN (8)..(8): Xaa is amino acid wherein carboxy group of asparatic acid is substituted with tetrazole
  MUTAGEN (17)..(17): Xaa is Nle
HSXGIFTXSYSRYRKQXAVKKYLAAVL

SEQ ID NO: 9 - protein, 27 aa, Artificial Sequence
  Syntehtic Peptide
  MUTAGEN (3)..(3): Xaa is amino acid wherein carboxy group of asparatic acid is substituted with tetrazole
  MUTAGEN (8)..(8): Xaa is amino acid wherein carboxy group of asparatic acid is substituted with tetrazole
HSXGIFTXSYSRYRKQLAVKKYLAAVL

SEQ ID NO: 10 - protein, 27 aa, Artificial Sequence
  Syntehtic Peptide
  MOD_RES (1)..(1): ACETYLATION
  MUTAGEN (3)..(3): Xaa is amino acid wherein carboxy group of asparatic acid is substituted with tetrazole
  MUTAGEN (8)..(8): Xaa is amino acid wherein carboxy group of asparatic acid is substituted with tetrazole
  MUTAGEN (17)..(17): Xaa is Nle
HSXGIFTXSYSRYRKQXAVKKYLAAVL

SEQ ID NO: 11 - protein, 27 aa, Artificial Sequence
  Syntehtic Peptide
  MOD_RES (1)..(1): ACETYLATION
  MUTAGEN (3)..(3): Xaa is amino acid wherein carboxy group of asparatic acid is substituted with tetrazole
  MUTAGEN (8)..(8): Xaa is amino acid wherein carboxy group of asparatic acid is substituted with tetrazole
HSXGIFTXSYSRYRKQLAVKKYLAAVL

SEQ ID NO: 12 - protein, 27 aa, Artificial Sequence
  Syntehtic Peptide
  MOD_RES (1)..(1): ACETYLATION
  MUTAGEN (3)..(3): Xaa is amino acid wherein carboxy group of asparatic acid is substituted with tetrazole
  MUTAGEN (8)..(8): Xaa is amino acid wherein carboxy group of asparatic acid is substituted with tetrazole
HSXGIFTXSYSRYRKQMAVKKYLAAVL

SEQ ID NO: 13 - protein, 27 aa, Artificial Sequence
  Syntehtic Peptide
  MOD_RES (1)..(1): Mesylation
  MUTAGEN (3)..(3): Xaa is amino acid wherein carboxy group of asparatic acid is substituted with tetrazole
  MUTAGEN (8)..(8): Xaa is amino acid wherein carboxy group of asparatic acid is substituted with tetrazole
  MUTAGEN (17)..(17): Xaa is Nle
HSXGIFTXSYSRYRKQXAVKKYLAAVL

SEQ ID NO: 14 - protein, 27 aa, Artificial Sequence
  Syntehtic Peptide
  MOD_RES (1)..(1): Mesylation
  MUTAGEN (3)..(3): Xaa is amino acid wherein carboxy group of asparatic acid is substituted with tetrazole
  MUTAGEN (8)..(8): Xaa is amino acid wherein carboxy group of asparatic acid is substituted with tetrazole
HSXGIFTXSYSRYRKQLAVKKYLAAVL

SEQ ID NO: 15 - protein, 27 aa, Artificial Sequence
  Synthetic peptide
  MOD_RES (1)..(1): ACETYLATION
  MUTAGEN (3)..(3): Xaa is amino acid wherein carboxy group of asparatic acid is substituted with tetrazole
  MUTAGEN (8)..(8): Xaa is amino acid wherein carboxy group of asparatic acid is substituted with tetrazole
  MUTAGEN (16)..(16): Xaa is amino acid wherein amide group of glutamine is substituted with tetrazole
HSXGIFTXSYSRYRKXLAVKKYLAAVL

SEQ ID NO: 16 - protein, 27 aa, Artificial Sequence
  Syntehtic Peptide
  MOD_RES (1)..(1): ACETYLATION
  MUTAGEN (3)..(3): Xaa is amino acid wherein carboxy group of asparatic acid is substituted with tetrazole
  MUTAGEN (8)..(8): Xaa is amino acid wherein carboxy group of asparatic acid is substituted with tetrazole
HAXGIFTXSYSRYRKQLAVKKYLAAVL

SEQ ID NO: 17 - protein, 27 aa, Artificial Sequence
  Syntehtic Peptide
  MOD_RES (1)..(1): ACETYLATION
  MUTAGEN (3)..(3): Xaa is amino acid wherein carboxy group of asparatic acid is substituted with tetrazole
  MUTAGEN (8)..(8): Xaa is amino acid wherein carboxy group of asparatic acid is substituted with tetrazole
HSXGIFTXAYSRYRKQLAVKKYLAAVL

SEQ ID NO: 18 - protein, 27 aa, Artificial Sequence
  Syntehtic Peptide
  MOD_RES (1)..(1): ACETYLATION
  MUTAGEN (3)..(3): Xaa is amino acid wherein carboxy group of asparatic acid is substituted with tetrazole
  MUTAGEN (8)..(8): Xaa is amino acid wherein carboxy group of asparatic acid is substituted with tetrazole
HSXGIFTXSYARYRKQLAVKKYLAAVL

SEQ ID NO: 19 - protein, 27 aa, Artificial Sequence
  Syntehtic Peptide
  MOD_RES (1)..(1): ACETYLATION
  MUTAGEN (3)..(3): Xaa is amino acid wherein carboxy group of asparatic acid is substituted with tetrazole
  MUTAGEN (8)..(8): Xaa is amino acid wherein carboxy group of asparatic acid is substituted with tetrazole
HSXGIFTXSYSRYRKALAVKKYLAAVL

SEQ ID NO: 20 - protein, 27 aa, Artificial Sequence
  Syntehtic Peptide
  MOD_RES (1)..(1): ACETYLATION
  MUTAGEN (3)..(3): Xaa is amino acid wherein carboxy group of asparatic acid is substituted with tetrazole
  MUTAGEN (8)..(8): Xaa is amino acid wherein carboxy group of asparatic acid is substituted with tetrazole
HSXGIFTXSYSRYRKQAAVKKYLAAVL

SEQ ID NO: 21 - protein, 27 aa, Artificial Sequence
  Syntehtic Peptide
  MOD_RES (1)..(1): ACETYLATION
  MUTAGEN (3)..(3): Xaa is amino acid wherein carboxy group of asparatic acid is substituted with tetrazole
  MUTAGEN (8)..(8): Xaa is amino acid wherein carboxy group of asparatic acid is substituted with tetrazole
HSXGIFTXSYSRYRKQLAAKKYLAAVL

SEQ ID NO: 22 - protein, 27 aa, Artificial Sequence
  Syntehtic Peptide
  MOD_RES (1)..(1): ACETYLATION
  MUTAGEN (3)..(3): Xaa is amino acid wherein carboxy group of asparatic acid is substituted with tetrazole
  MUTAGEN (8)..(8): Xaa is amino acid wherein carboxy group of asparatic acid is substituted with tetrazole
HSXGIFTXSYSRYRKQLAVKKYLAAVA

SEQ ID NO: 23 - protein, 27 aa, Artificial Sequence
  Syntehtic Peptide
  MOD_RES (1)..(1): ACETYLATION
  MUTAGEN (3)..(3): Xaa is amino acid wherein carboxy group of asparatic acid is substituted with tetrazole
  MUTAGEN (8)..(8): Xaa is amino acid wherein carboxy group of asparatic acid is substituted with tetrazole
HSXGIFTXSYSRYRRQLAVRRYLAAVL

SEQ ID NO: 24 - protein, 30 aa, Artificial Sequence
  Syntehtic Peptide
  MOD_RES (1)..(1): ACETYLATION
  MUTAGEN (3)..(3): Xaa is amino acid wherein carboxy group of asparatic acid is substituted with tetrazole
  MUTAGEN (8)..(8): Xaa is amino acid wherein carboxy group of asparatic acid is substituted with tetrazole
HSXGIFTXSYSRYRRQLAVRRYLAAVLGRR

SEQ ID NO: 25 - protein, 27 aa, Artificial Sequence
  Syntehtic Peptide
  MOD_RES (1)..(1): ACETYLATION
  MUTAGEN (3)..(3): Xaa is amino acid wherein carboxy group of asparatic acid is substituted with tetrazole
  MUTAGEN (8)..(8): Xaa is amino acid wherein carboxy group of asparatic acid is substituted with tetrazole
HSXAIFTXSYSRYRKQLAVKKYLAAVL

SEQ ID NO: 26 - protein, 27 aa, Artificial Sequence
  Syntehtic Peptide
  MOD_RES (1)..(1): ACETYLATION
  MUTAGEN (3)..(3): Xaa is amino acid wherein carboxy group of asparatic acid is substituted with tetrazole
  MUTAGEN (8)..(8): Xaa is amino acid wherein carboxy group of asparatic acid is substituted with tetrazole
HAXGIFTXAYSRYRKQLAVKKYLAAVL

SEQ ID NO: 27 - protein, 27 aa, Artificial Sequence
  Syntehtic Peptide
  MOD_RES (1)..(1): ACETYLATION
  MUTAGEN (3)..(3): Xaa is amino acid wherein carboxy group of asparatic acid is substituted with tetrazole
  MUTAGEN (8)..(8): Xaa is amino acid wherein carboxy group of asparatic acid is substituted with tetrazole
HAXGIFTXSYSRYRKQAAVKKYLAAVL

SEQ ID NO: 28 - protein, 27 aa, Artificial Sequence
  Syntehtic Peptide
  MOD_RES (1)..(1): ACETYLATION
  MUTAGEN (3)..(3): Xaa is amino acid wherein carboxy group of asparatic acid is substituted with tetrazole
  MUTAGEN (8)..(8): Xaa is amino acid wherein carboxy group of asparatic acid is substituted with tetrazole
HSXGIFTXAYSRYRKALAVKKYLAAVL

SEQ ID NO: 29 - protein, 27 aa, Artificial Sequence
  Syntehtic Peptide
  MOD_RES (1)..(1): ACETYLATION
  MUTAGEN (3)..(3): Xaa is amino acid wherein carboxy group of asparatic acid is substituted with tetrazole
  MUTAGEN (8)..(8): Xaa is amino acid wherein carboxy group of asparatic acid is substituted with tetrazole
HSXGIFTXAYSRYRKQAAVKKYLAAVL

SEQ ID NO: 30 - protein, 27 aa, Artificial Sequence
  Syntehtic Peptide
  MOD_RES (1)..(1): ACETYLATION
  MUTAGEN (3)..(3): Xaa is amino acid wherein carboxy group of asparatic acid is substituted with tetrazole
  MUTAGEN (8)..(8): Xaa is amino acid wherein carboxy group of asparatic acid is substituted with tetrazole
HSXGIFTXSYSRYRKAAAVKKYLAAVL

SEQ ID NO: 31 - protein, 27 aa, Artificial Sequence
  Syntehtic Peptide
  MOD_RES (1)..(1): Mesylation
  MUTAGEN (3)..(3): Xaa is amino acid wherein carboxy group of asparatic acid is substituted with tetrazole
  MUTAGEN (8)..(8): Xaa is amino acid wherein carboxy group of asparatic acid is substituted with tetrazole
HSXGIFTXAYSRYRKQLAVKKYLAAVL

SEQ ID NO: 32 - protein, 27 aa, Artificial Sequence
  Syntehtic Peptide
  MOD_RES (1)..(1): Mesylation
  MUTAGEN (3)..(3): Xaa is amino acid wherein carboxy group of asparatic acid is substituted with tetrazole
  MUTAGEN (8)..(8): Xaa is amino acid wherein carboxy group of asparatic acid is substituted with tetrazole
HSXAIFTXSYSRYRKQLAVKKYLAAVL

SEQ ID NO: 33 - protein, 27 aa, Artificial Sequence
  Syntehtic Peptide
  MOD_RES (1)..(1): Mesylation
  MUTAGEN (3)..(3): Xaa is amino acid wherein carboxy group of asparatic acid is substituted with tetrazole
  MUTAGEN (8)..(8): Xaa is amino acid wherein carboxy group of asparatic acid is substituted with tetrazole
HSXAIFTXSYSRYRKQAAVKKYLAAVL

SEQ ID NO: 34 - protein, 27 aa, Artificial Sequence
  Syntehtic Peptide
  MOD_RES (1)..(1): ACETYLATION
  MUTAGEN (3)..(3): Xaa is amino acid wherein carboxy group of asparatic acid is substituted with tetrazole
  MUTAGEN (8)..(8): Xaa is amino acid wherein carboxy group of asparatic acid is substituted with tetrazole
HSXAIFTXSYSRYRKQAAVKKYLAAVL

SEQ ID NO: 35 - protein, 27 aa, Artificial Sequence
  Syntehtic Peptide
  MOD_RES (1)..(1): ACETYLATION
  MUTAGEN (3)..(3): Xaa is amino acid wherein carboxy group of asparatic acid is substituted with tetrazole
  MUTAGEN (8)..(8): Xaa is amino acid wherein carboxy group of asparatic acid is substituted with tetrazole
HAXAIFTXSYSRYRKQAAVKKYLAAVL

SEQ ID NO: 36 - protein, 27 aa, Artificial Sequence
  Syntehtic Peptide
  MOD_RES (1)..(1): ACETYLATION
  MUTAGEN (3)..(3): Xaa is amino acid wherein carboxy group of asparatic acid is substituted with tetrazole
  MUTAGEN (8)..(8): Xaa is amino acid wherein carboxy group of asparatic acid is substituted with tetrazole
HSXAIFTXSYSRYRKAAAVKKYLAAVL

SEQ ID NO: 37 - protein, 11 aa, Artificial Sequence
  Synthetic peptide
GKRYKQRVKNK

SEQ ID NO: 38 - protein, 10 aa, Artificial Sequence
  Synthetic peptide
GKRYKQRVKN

SEQ ID NO: 39 - protein, 9 aa, Artificial Sequence
  Synthetic peptide
GKRYKQRVK

SEQ ID NO: 40 - protein, 8 aa, Artificial Sequence
  Synthetic peptide
GKRYKQRV

SEQ ID NO: 41 - protein, 7 aa, Artificial Sequence
  Synthetic peptide
GKRYKQR

SEQ ID NO: 42 - protein, 6 aa, Artificial Sequence
  Synthetic peptide
GKRYKQ

SEQ ID NO: 43 - protein, 5 aa, Artificial Sequence
  Synthetic peptide
GKRYK

SEQ ID NO: 44 - protein, 4 aa, Artificial Sequence
  Synthetic peptide
GKRY